European Patent Specification EP 3 608 338 B1, published March 11, 2026. Title: Human Antibodies to the Glucagon Receptor. Applicant: Regeneron Pharmaceuticals, Inc. Application To be assigned. The sequence listing filed with the application follows.

SEQUENCE LISTING (207 sequences)

SEQ ID NO: 1 - DNA, 375 bp, Artificial Sequence
  Synthetic
caggtccagttggtacagtctggggctgacgtgaagaagcctggggcctcagtgaaggtctcctgcaaggtttccggacatatcctcactgatttatccatgcactgggtgcgacagcctcctggaaaaggacttgagtggatggcaggttttgatcctgaagaaggtaaaataatctacgcacagaagttccagggcagagtcaccatgaccgaggacacatctacagacacagcctacatggagctgagcagcctgagatctggggacacggccgtttattactgtgcaacaagcgatattttgactgggtattatagagactactacggtttggacgtctggggccaagggaccacgctcaccgtctcctca

SEQ ID NO: 2 - protein, 125 aa, Artificial Sequence
  Synthetic
QVQLVQSGADVKKPGASVKVSCKVSGHILTDLSMHWVRQPPGKGLEWMAGFDPEEGKIIYAQKFQGRVTMTEDTSTDTAYMELSSLRSGDTAVYYCATSDILTGYYRDYYGLDVWGQGTTLTVSS

SEQ ID NO: 3 - DNA, 24 bp, Artificial Sequence
  Synthetic
ggacatatcctcactgatttatcc

SEQ ID NO: 4 - protein, 8 aa, Artificial Sequence
  Synthetic
GHILTDLS

SEQ ID NO: 5 - DNA, 24 bp, Artificial Sequence
  Synthetic
tttgatcctgaagaaggtaaaata

SEQ ID NO: 6 - protein, 8 aa, Artificial Sequence
  Synthetic
FDPEEGKI

SEQ ID NO: 7 - DNA, 54 bp, Artificial Sequence
  Synthetic
gcaacaagcgatattttgactgggtattatagagactactacggtttggacgtc

SEQ ID NO: 8 - protein, 18 aa, Artificial Sequence
  Synthetic
ATSDILTGYYRDYYGLDV

SEQ ID NO: 9 - DNA, 336 bp, Artificial Sequence
  Synthetic
gatattgtgatgactcagtctccactcttcctgcccgtcacccctggagagccggcctccatctcctgcaggtctagtcagagcctcctgcatagtaaaggatacaactatttggattggtacctgcagaagccagggcagtctccacaactcctgatctatttgggttctaatcgggcctccggggtccctgacaggttcagtggcagtggatcaggcacagattttacactgaaaatcagcagagtggaggctgaagatgttggggtttattactgcatgcaaactctacaaactcctcggacgttcggccaagggaccaaggtggaaatcaaa

SEQ ID NO: 10 - protein, 112 aa, Artificial Sequence
  Synthetic
DIVMTQSPLFLPVTPGEPASISCRSSQSLLHSKGYNYLDWYLQKPGQSPQLLIYLGSNRASGVPDRFSGSGSGTDFTLKISRVEAEDVGVYYCMQTLQTPRTFGQGTKVEIK

SEQ ID NO: 11 - DNA, 33 bp, Artificial Sequence
  Synthetic
cagagcctcctgcatagtaaaggatacaactat

SEQ ID NO: 12 - protein, 11 aa, Artificial Sequence
  Synthetic
QSLLHSKGYNY

SEQ ID NO: 13 - DNA, 9 bp, Artificial Sequence
  Synthetic
ttgggttct

SEQ ID NO: 14 - protein, 3 aa, Artificial Sequence
  Synthetic
LGS

SEQ ID NO: 15 - DNA, 27 bp, Artificial Sequence
  Synthetic
atgcaaactctacaaactcctcggacg

SEQ ID NO: 16 - protein, 9 aa, Artificial Sequence
  Synthetic
MQTLQTPRT

SEQ ID NO: 17 - DNA, 375 bp, Artificial Sequence
  Synthetic
caggtccagttggtacagtctggggctgacgtgaagaagcctggggcctcagtgaaggtctcctgcaaggtttccggacatatcctcactgatttatccatgcactgggtgcgacaggctcctggaaaagggcttgagtggatgggaggttttgatcctgaagaaggtgaaataatctacgcacagaagttccagggcagagtcaccatgaccgaggacacatctacagacacagcctacatggagctgagcagcctgagatctggggacacggccgtttattactgtgcaacaagcgatattttgactggttattatagagactactacggtttggacgtctggggccaagggaccacgctcaccgtctcctca

SEQ ID NO: 18 - protein, 125 aa, Artificial Sequence
  Synthetic
QVQLVQSGADVKKPGASVKVSCKVSGHILTDLSMHWVRQAPGKGLEWMGGFDPEEGEIIYAQKFQGRVTMTEDTSTDTAYMELSSLRSGDTAVYYCATSDILTGYYRDYYGLDVWGQGTTLTVSS

SEQ ID NO: 19 - DNA, 24 bp, Artificial Sequence
  Synthetic
ggacatatcctcactgatttatcc

SEQ ID NO: 20 - protein, 8 aa, Artificial Sequence
  Synthetic
GHILTDLS

SEQ ID NO: 21 - DNA, 24 bp, Artificial Sequence
  Synthetic
tttgatcctgaagaaggtgaaata

SEQ ID NO: 22 - protein, 8 aa, Artificial Sequence
  Synthetic
FDPEEGEI

SEQ ID NO: 23 - DNA, 54 bp, Artificial Sequence
  Synthetic
gcaacaagcgatattttgactggttattatagagactactacggtttggacgtc

SEQ ID NO: 24 - protein, 18 aa, Artificial Sequence
  Synthetic
ATSDILTGYYRDYYGLDV

SEQ ID NO: 25 - DNA, 336 bp, \Artificial Sequence; identical to SEQ ID NO: 9
  Synthetic

SEQ ID NO: 26 - protein, 112 aa, Artificial Sequence; identical to SEQ ID NO: 10
  Synthetic

SEQ ID NO: 27 - DNA, 33 bp, Artificial Sequence; identical to SEQ ID NO: 11
  Synthetic

SEQ ID NO: 28 - protein, 11 aa, Artificial Sequence
  Synthetic
QSLLHSKGYNY

SEQ ID NO: 29 - DNA, 9 bp, Artificial Sequence
  Synthetic
ttgggttct

SEQ ID NO: 30 - protein, 3 aa, Artificial Sequence
  Synthetic
LGS

SEQ ID NO: 31 - DNA, 27 bp, Artificial Sequence
  Synthetic
atgcaaactctacaaactcctcggacg

SEQ ID NO: 32 - protein, 9 aa, Artificial Sequence
  Synthetic
MQTLQTPRT

SEQ ID NO: 33 - DNA, 372 bp, Artificial Sequence
  Synthetic
gaggagcaactggtggagtctgggggagacttggtacagcctggagggtccctaagactctcctgtgcagcctctggattcactctcagtagttatgaaatgaactgggtccgccaggctccagggaaggggctggagtgggtttcatacattagtagaggtggtagtctgatacactacacagactctgtgaagggccgattcaccatctccagagacaacgccaagaattcactgtatctgcaaatgaacagcctgagagccgaggacacggctgtttattactgtgtgagagacccagcagctcgttatcattattattatcacggtatggacgtctggggccaagggaccacggtcaccgtctcctca

SEQ ID NO: 34 - protein, 124 aa, Artificial Sequence
  Synthetic
EEQLVESGGDLVQPGGSLRLSCAASGFTLSSYEMNWVRQAPGKGLEWVSYISRGGSLIHYTDSVKGRFTISRDNAKNSLYLQMNSLRAEDTAVYYCVRDPAARYHYYYHGMDVWGQGTTVTVSS

SEQ ID NO: 35 - DNA, 24 bp, Artificial Sequence
  Synthetic
ggattcactctcagtagttatgaa

SEQ ID NO: 36 - protein, 8 aa, Artificial Sequence
  Synthetic
GFTLSSYE

SEQ ID NO: 37 - DNA, 24 bp, Artificial Sequence
  Synthetic
attagtagaggtggtagtctgata

SEQ ID NO: 38 - protein, 8 aa, Artificial Sequence
  Synthetic
ISRGGSLI

SEQ ID NO: 39 - DNA, 51 bp, Artificial Sequence
  Synthetic
gtgagagacccagcagctcgttatcattattattatcacggtatggacgtc

SEQ ID NO: 40 - protein, 17 aa, Artificial Sequence
  Synthetic
VRDPAARYHYYYHGMDV

SEQ ID NO: 41 - DNA, 336 bp, Artificial Sequence
  Synthetic
gatattgtgatgactcagtctccactctccctgcccgtcacccctggagagccggcctccatctcctgcaggtctagtcagagcctcctgcacaataatggatataactatttggattggtatctgcagaagccagggcagtctccacagctcctgatctatttgggttctagtcgggcctccggggtccctgacaggttcagtggcagtggatcaggcacagattttatactgaaaatcagcagagtggaggctgaagatgttggggtttattactgcatgcaagctctacaaactccgtggacgttcggccgagggaccaaggtggaaatcaaa

SEQ ID NO: 42 - protein, 112 aa, Artificial Sequence
  Synthetic
DIVMTQSPLSLPVTPGEPASISCRSSQSLLHNNGYNYLDWYLQKPGQSPQLLIYLGSSRASGVPDRFSGSGSGTDFILKISRVEAEDVGVYYCMQALQTPWTFGRGTKVEIK

SEQ ID NO: 43 - DNA, 33 bp, Artificial Sequence
  Synthetic
cagagcctcctgcacaataatggatataactat

SEQ ID NO: 44 - protein, 11 aa, Artificial Sequence
  Synthetic
QSLLHNNGYNY

SEQ ID NO: 45 - DNA, 9 bp, Artificial Sequence
  Synthetic
ttgggttct

SEQ ID NO: 46 - protein, 3 aa, Artificial Sequence
  Synthetic
LGS

SEQ ID NO: 47 - DNA, 27 bp, Artificial Sequence
  Synthetic
atgcaagctctacaaactccgtggacg

SEQ ID NO: 48 - protein, 9 aa, Artificial Sequence
  Synthetic
MQALQTPWT

SEQ ID NO: 49 - DNA, 384 bp, Artificial Sequence
  Synthetic
gaggtgcagctggtggagtctgggggaggcgtggtccagcctgggaggtccctgagactctcctgtgcagcctctggattcaccttcagtagttatgacatgcactgggtccgccaggctccaggcaaggggctggagtgggtggcagttatatcatctgatggacgtgataaatactatgtagactccgtgaagggccgattcaccatctccagagacaactccaagaacacgctttatctgcaaatgaacagcctgagagctgaggacacggctgtttattactgtgcgaaagagatggtgtattacgatattttgactggttatcataactactacggtatggacgtctggggccaagggaccacggtcaccgtctcctca

SEQ ID NO: 50 - protein, 128 aa, Artificial Sequence
  Synthetic
EVQLVESGGGVVQPGRSLRLSCAASGFTFSSYDMHWVRQAPGKGLEWVAVISSDGRDKYYVDSVKGRFTISRDNSKNTLYLQMNSLRAEDTAVYYCAKEMVYYDILTGYHNYYGMDVWGQGTTVTVSS

SEQ ID NO: 51 - DNA, 24 bp, Artificial Sequence
  Synthetic
ggattcaccttcagtagttatgac

SEQ ID NO: 52 - protein, 8 aa, Artificial Sequence
  Synthetic
GFTFSSYD

SEQ ID NO: 53 - DNA, 24 bp, Artificial Sequence
  Synthetic
atatcatctgatggacgtgataaa

SEQ ID NO: 54 - protein, 8 aa, Artificial Sequence
  Synthetic
ISSDGRDK

SEQ ID NO: 55 - DNA, 63 bp, Artificial Sequence
  Synthetic
gcgaaagagatggtgtattacgatattttgactggttatcataactactacggtatggacgtc

SEQ ID NO: 56 - protein, 21 aa, Artificial Sequence
  Synthetic
AKEMVYYDILTGYHNYYGMDV

SEQ ID NO: 57 - DNA, 324 bp, Artificial Sequence
  Synthetic
gacatcgtgatgacccagtctccatcctcactgtctgcatctgtaggagacagagtcaccatcacttgtcgggcgagtcagggcattaacaattatttagcctggtttcagcagaaaccagggaaagcccctaagtccctgatccatactgcatccagtttgcaaagtggggtcccatcaaagttcagcggcagtggatctgggacagatttcactctcaccatcagcagcctgcagcctgaagattttgcaacttattactgccaacagtataatacttaccctctcactttcggcggagggaccaaagtggagatcaaacga

SEQ ID NO: 58 - protein, 108 aa, \Artificial Sequence
  Synthetic
DIVMTQSPSSLSASVGDRVTITCRASQGINNYLAWFQQKPGKAPKSLIHTASSLQSGVPSKFSGSGSGTDFTLTISSLQPEDFATYYCQQYNTYPLTFGGGTKVEIKR

SEQ ID NO: 59 - DNA, 18 bp, Artificial Sequence
  Synthetic
cagggcattaacaattat

SEQ ID NO: 60 - protein, 6 aa, Artificial Sequence
  Synthetic
QGINNY

SEQ ID NO: 61 - DNA, 9 bp, Artificial Sequence
  Synthetic
actgcatcc

SEQ ID NO: 62 - protein, 3 aa, Artificial Sequence
  Synthetic
TAS

SEQ ID NO: 63 - DNA, 27 bp, Artificial Sequence
  Synthetic
caacagtataatacttaccctctcact

SEQ ID NO: 64 - protein, 9 aa, Artificial Sequence
  Synthetic
QQYNTYPLT

SEQ ID NO: 65 - DNA, 381 bp, Artificial Sequence
  Synthetic
caggtgcagctggtggagtctgggggaggcgtggtccagcctgggaggtccctgagactctcctgtgcagcctctggattcaccttcagtagttatgacatgcactgggtccgccaggctccaggcaaggggctggagtgggtggcagttatatcatctgatggacgtgataaatactatgtagactccgtgaagggccgattcaccatctccagagacaactccaagaacacgctttatctgcaaatgaacagcctgagagctgaggacacggctgtttattactgtgcgaaagagatggtgtattacgatattttgactggttatcataactactacggtatggacgtctggggccaagggaccacggtcaccgtctcc

SEQ ID NO: 66 - protein, 127 aa, Artificial Sequence
  Synthetic
QVQLVESGGGVVQPGRSLRLSCAASGFTFSSYDMHWVRQAPGKGLEWVAVISSDGRDKYYVDSVKGRFTISRDNSKNTLYLQMNSLRAEDTAVYYCAKEMVYYDILTGYHNYYGMDVWGQGTTVTVS

SEQ ID NO: 67 - DNA, 321 bp, Artificial Sequence
  Synthetic
gacatccagatgacccagtctccatcctcactgtctgcatctgtaggagacagagtcaccatcacttgtcgggcgagtcagggcattaacaattatttagcctggtttcagcagaaaccagggaaagcccctaagtccctgatccatactgcatccagtttgcaaagtggggtcccatcaaagttcagcggcagtggatctgggacagatttcactctcaccatcagcagcctgcagcctgaagattttgcaacttattactgccaacagtataatacttaccctctcactttcggcggagggaccaaggtggagatcaaa

SEQ ID NO: 68 - protein, 107 aa, Artificial Sequence
  Synthetic
DIQMTQSPSSLSASVGDRVTITCRASQGINNYLAWFQQKPGKAPKSLIHTASSLQSGVPSKFSGSGSGTDFTLTISSLQPEDFATYYCQQYNTYPLTFGGGTKVEIK

SEQ ID NO: 69 - DNA, 384 bp, Artificial Sequence
  Synthetic
caggtgcagctggtgcagtctgggggaggcttggtccagcctggggggtccctgagactctcctgtgcagcctccggattcacctttagtaactatttgatgaactgggtccgccaggctccagggaaggggctggagtggctggccaacatacaggaagatggaattgagaaatactatgtggactctgtgaagggccgattcaccatctccagagacaacgccaagaactcactgtatctgcaaatgaacagcctgagagccgaggacacggctgtgtattactgtgcgagagagccctcccattacgatattttgactggttatgactactattacggtatggacgtctggggccaagggaccacggtcaccgtctcctca

SEQ ID NO: 70 - protein, 128 aa, Artificial Sequence
  Synthetic
QVQLVQSGGGLVQPGGSLRLSCAASGFTFSNYLMNWVRQAPGKGLEWLANIQEDGIEKYYVDSVKGRFTISRDNAKNSLYLQMNSLRAEDTAVYYCAREPSHYDILTGYDYYYGMDVWGQGTTVTVSS

SEQ ID NO: 71 - DNA, 24 bp, Artificial Sequence
  Synthetic
ggattcacctttagtaactatttg

SEQ ID NO: 72 - protein, 8 aa, Artificial Sequence
  Synthetic
GFTFSNYL

SEQ ID NO: 73 - DNA, 24 bp, Artificial Sequence
  Synthetic
atacaggaagatggaattgagaaa

SEQ ID NO: 74 - protein, 8 aa, Artificial Sequence
  Synthetic
IQEDGIEK

SEQ ID NO: 75 - DNA, 63 bp, Artificial Sequence
  Synthetic
gcgagagagccctcccattacgatattttgactggttatgactactattacggtatggacgtc

SEQ ID NO: 76 - protein, 21 aa, Artificial Sequence
  Synthetic
AREPSHYDILTGYDYYYGMDV

SEQ ID NO: 77 - DNA, 324 bp, Artificial Sequence
  Synthetic
gacatccagttgacccagtctccatcctccctgtctgcatctgtaggagacagagtcaccatcacttgccgggcaagtcagggcattagaaatgatttaggctggtatcagcagaaaccagggaaagcccctaagcgcctgatctatgctgcatccagtttgcaaagtggggtcccatcaaggttcagcggcagtggatctgggacagaattcattctcacagtcagcagcctgcagcctgaagactttgcaacttattactgtctacagtataatagtaacccattcactttcggccctgggaccaaggtggagatcaaacga

SEQ ID NO: 78 - protein, 108 aa, Artificial Sequence
  Synthetic
DIQLTQSPSSLSASVGDRVTITCRASQGIRNDLGWYQQKPGKAPKRLIYAASSLQSGVPSRFSGSGSGTEFILTVSSLQPEDFATYYCLQYNSNPFTFGPGTKVEIKR

SEQ ID NO: 79 - DNA, 18 bp, Artificial Sequence
  Synthetic
cagggcattagaaatgat

SEQ ID NO: 80 - protein, 6 aa, Artificial Sequence
  Synthetic
QGIRND

SEQ ID NO: 81 - DNA, 9 bp, Artificial Sequence
  Synthetic
gctgcatcc

SEQ ID NO: 82 - protein, 3 aa, Artificial Sequence
  Synthetic
AAS

SEQ ID NO: 83 - DNA, 27 bp, Artificial Sequence
  Synthetic
ctacagtataatagtaacccattcact

SEQ ID NO: 84 - protein, 9 aa, Artificial Sequence
  Synthetic
LQYNSNPFT

SEQ ID NO: 85 - DNA, 381 bp, Artificial Sequence
  Synthetic
gaggtgcagctggtggagtctgggggaggcttggtccagcctggggggtccctgagactctcctgtgcagcctccggattcacctttagtaactatttgatgaactgggtccgccaggctccagggaaggggctggagtggctggccaacatacaggaagatggaattgagaaatactatgtggactctgtgaagggccgattcaccatctccagagacaacgccaagaactcactgtatctgcaaatgaacagcctgagagccgaggacacggctgtgtattactgtgcgagagagccctcccattacgatattttgactggttatgactactattacggtatggacgtctggggccaagggaccacggtcaccgtctcc

SEQ ID NO: 86 - protein, 127 aa, Artificial Sequence
  Synthetic
EVQLVESGGGLVQPGGSLRLSCAASGFTFSNYLMNWVRQAPGKGLEWLANIQEDGIEKYYVDSVKGRFTISRDNAKNSLYLQMNSLRAEDTAVYYCAREPSHYDILTGYDYYYGMDVWGQGTTVTVS

SEQ ID NO: 87 - DNA, 321 bp, Artificial Sequence
  Synthetic
gacatccagatgacccagtctccatcctccctgtctgcatctgtaggagacagagtcaccatcacttgccgggcaagtcagggcattagaaatgatttaggctggtatcagcagaaaccagggaaagcccctaagcgcctgatctatgctgcatccagtttgcaaagtggggtcccatcaaggttcagcggcagtggatctgggacagaattcattctcacagtcagcagcctgcagcctgaagactttgcaacttattactgtctacagtataatagtaacccattcactttcggccctgggaccaaagtggatatcaaa

SEQ ID NO: 88 - protein, 107 aa, Artificial Sequence
  Synthetic
DIQMTQSPSSLSASVGDRVTITCRASQGIRNDLGWYQQKPGKAPKRLIYAASSLQSGVPSRFSGSGSGTEFILTVSSLQPEDFATYYCLQYNSNPFTFGPGTKVDIK

SEQ ID NO: 89 - DNA, 381 bp, Artificial Sequence
  Synthetic
gaggtgcagctggtgcagtctgggggagccttggtacagcctggggggtccctgagactctcctgtacagcctctggtttcaccttcagtaactacgacatgcactgggtccgccaaactacaggaaaaggtctggagtggatctcagctattgatactgctggtgacacatactatccaggctccgtgaagggccgattcaccgtctccagagaaaatgccaagaactccttttatcttcaaatgaacagcctgagagccggggacacggctgtgtattactgtgcaagggaggggaagtattacgatattttgactggtgactaccactactacggtatggacgtctggggccaagggaccacggtcaccgtctcctca

SEQ ID NO: 90 - protein, 127 aa, Artificial Sequence
  Synthetic
EVQLVQSGGALVQPGGSLRLSCTASGFTFSNYDMHWVRQTTGKGLEWISAIDTAGDTYYPGSVKGRFTVSRENAKNSFYLQMNSLRAGDTAVYYCAREGKYYDILTGDYHYYGMDVWGQGTTVTVSS

SEQ ID NO: 91 - DNA, 24 bp, Artificial Sequence
  Synthetic
ggtttcaccttcagtaactacgac

SEQ ID NO: 92 - protein, 8 aa, Artificial Sequence
  Synthetic
GFTFSNYD

SEQ ID NO: 93 - DNA, 21 bp, Artificial Sequence
  Synthetic
attgatactgctggtgacaca

SEQ ID NO: 94 - protein, 7 aa, Artificial Sequence
  Synthetic
IDTAGDT

SEQ ID NO: 95 - DNA, 63 bp, Artificial Sequence
  Synthetic
gcaagggaggggaagtattacgatattttgactggtgactaccactactacggtatggacgtc

SEQ ID NO: 96 - protein, 21 aa, Artificial Sequence
  Synthetic
AREGKYYDILTGDYHYYGMDV

SEQ ID NO: 97 - DNA, 324 bp, Artificial Sequence
  Synthetic
gccatccggatgacccagtctccatcctccctgtctgcatctgtaggagacagagtcaccatcacttgtcgggcaagtcagggcattagaaatgatttaggctggtatcagcagaaaccagggaaagcccctaagcgactgatctatgctacatccagtttgcaaagtggggtcccatcaaggttcagcggcagtggatctgggacagaattcactctcacaatcagcagcctgcagcctgaagattttgcaacttattactgtctacagcataatagttacccgctcactttcggcggagggaccaaggtggaaatcaaacga

SEQ ID NO: 98 - protein, 108 aa, Artificial Sequence
  Synthetic
AIRMTQSPSSLSASVGDRVTITCRASQGIRNDLGWYQQKPGKAPKRLIYATSSLQSGVPSRFSGSGSGTEFTLTISSLQPEDFATYYCLQHNSYPLTFGGGTKVEIKR

SEQ ID NO: 99 - DNA, 18 bp, Artificial Sequence
  Synthetic
cagggcattagaaatgat

SEQ ID NO: 100 - protein, 6 aa, Artificial Sequence
  Synthetic
QGIRND

SEQ ID NO: 101 - DNA, 9 bp, Artificial Sequence
  Synthetic
gctacatcc

SEQ ID NO: 102 - protein, 3 aa, Artificial Sequence
  Synthetic
ATS

SEQ ID NO: 103 - DNA, 27 bp, Artificial Sequence
  Synthetic
ctacagcataatagttacccgctcact

SEQ ID NO: 104 - protein, 9 aa, Artificial Sequence
  Synthetic
LQHNSYPLT

SEQ ID NO: 105 - DNA, 378 bp, Artificial Sequence
  Synthetic
gaggtgcagctggtggagtctgggggagccttggtacagcctggggggtccctgagactctcctgtacagcctctggtttcaccttcagtaactacgacatgcactgggtccgccaaactacaggaaaaggtctggagtggatctcagctattgatactgctggtgacacatactatccaggctccgtgaagggccgattcaccgtctccagagaaaatgccaagaactccttttatcttcaaatgaacagcctgagagccggggacacggctgtgtattactgtgcaagggaggggaagtattacgatattttgactggtgactaccactactacggtatggacgtctggggccaagggaccacggtcaccgtctcc

SEQ ID NO: 106 - protein, 126 aa, Artificial Sequence
  Synthetic
EVQLVESGGALVQPGGSLRLSCTASGFTFSNYDMHWVRQTTGKGLEWISAIDTAGDTYYPGSVKGRFTVSRENAKNSFYLQMNSLRAGDTAVYYCAREGKYYDILTGDYHYYGMDVWGQGTTVTVS

SEQ ID NO: 107 - DNA, 321 bp, Artificial Sequence
  Synthetic
gacatccagatgacccagtctccatcctccctgtctgcatctgtaggagacagagtcaccatcacttgtcgggcaagtcagggcattagaaatgatttaggctggtatcagcagaaaccagggaaagcccctaagcgactgatctatgctacatccagtttgcaaagtggggtcccatcaaggttcagcggcagtggatctgggacagaattcactctcacaatcagcagcctgcagcctgaagattttgcaacttattactgtctacagcataatagttacccgctcactttcggcggagggaccaagctggagatcaaa

SEQ ID NO: 108 - protein, 107 aa, Artificial Sequence
  Synthetic
DIQMTQSPSSLSASVGDRVTITCRASQGIRNDLGWYQQKPGKAPKRLIYATSSLQSGVPSRFSGSGSGTEFTLTISSLQPEDFATYYCLQHNSYPLTFGGGTKLEIK

SEQ ID NO: 109 - DNA, 372 bp, Artificial Sequence
  Synthetic
caggtgcagctggtgcagtctgggggaggcgtggtccagcctgggaggtccctgagactctcctgtgcagcgtctgggttcacctttagtaactttggcatgcactgggtccgccaggctccaggcaaggggctggagtgggtggcagttatatggtttgatgaaattgataaatactatgcagactccgtgaagggccgattcaccatctccagagacaattccaagaacacgctgtatccgcaaatgaacagcctgagagccgaagacacggctgtgtattactgtgcgcgagaagattacgatattttgactggttactattacgctatggacgtctggggccaagggaccacggtcaccgtctcctca

SEQ ID NO: 110 - protein, 124 aa, Artificial Sequence
  Synthetic
QVQLVQSGGGVVQPGRSLRLSCAASGFTFSNFGMHWVRQAPGKGLEWVAVIWFDEIDKYYADSVKGRFTISRDNSKNTLYPQMNSLRAEDTAVYYCAREDYDILTGYYYAMDVWGQGTTVTVSS

SEQ ID NO: 111 - DNA, 24 bp, Artificial Sequence
  Synthetic
gggttcacctttagtaactttggc

SEQ ID NO: 112 - protein, 8 aa, Artificial Sequence
  Synthetic
GFTFSNFG

SEQ ID NO: 113 - DNA, 24 bp, Artificial Sequence
  Synthetic
atatggtttgatgaaattgataaa

SEQ ID NO: 114 - protein, 8 aa, Artificial Sequence
  Synthetic
IWFDEIDK

SEQ ID NO: 115 - DNA, 51 bp, Artificial Sequence
  Synthetic
gcgcgagaagattacgatattttgactggttactattacgctatggacgtc

SEQ ID NO: 116 - protein, 17 aa, Artificial Sequence
  Synthetic
AREDYDILTGYYYAMDV

SEQ ID NO: 117 - DNA, 321 bp, Artificial Sequence
  Synthetic
gacatccagatgacccagtctccatcctccctgtctgcatctgtaggagacagagtcaccatcacttgccgggcaagtcagggcattagaaatgatttaggctggtatcagcagaaaccagggaaagcccctaagcgcctaatctatgctgcatcccgtttgcaaagtggggtcccatcgaggttcagcggcagtggatctgggacagaattcactctcacaatcagcagcctgcagcctgaagattttggaacttattactgtctacagcataatagtcaccccaccttcggccaagggaccaaggtggagatcaaacga

SEQ ID NO: 118 - protein, 107 aa, Artificial Sequence
  Synthetic
DIQMTQSPSSLSASVGDRVTITCRASQGIRNDLGWYQQKPGKAPKRLIYAASRLQSGVPSRFSGSGSGTEFTLTISSLQPEDFGTYYCLQHNSHPTFGQGTKVEIKR

SEQ ID NO: 119 - DNA, 18 bp, Artificial Sequence
  Synthetic
cagggcattagaaatgat

SEQ ID NO: 120 - protein, 6 aa, Artificial Sequence
  Synthetic
QGIRND

SEQ ID NO: 121 - DNA, 9 bp, Artificial Sequence
  Synthetic
gctgcatcc

SEQ ID NO: 122 - protein, 3 aa, Artificial Sequence
  Synthetic
AAS

SEQ ID NO: 123 - DNA, 24 bp, Artificial Sequence
  Synthetic
ctacagcataatagtcaccccacc

SEQ ID NO: 124 - protein, 8 aa, Artificial Sequence
  Synthetic
LQHNSHPT

SEQ ID NO: 125 - DNA, 369 bp, Artificial Sequence
  Synthetic
caggtgcagctggtggagtctgggggaggcgtggtccagcctgggaggtccctgagactctcctgtgcagcgtctgggttcacctttagtaactttggcatgcactgggtccgccaggctccaggcaaggggctggagtgggtggcagttatatggtttgatgaaattgataaatactatgcagactccgtgaagggccgattcaccatctccagagacaattccaagaacacgctgtatccgcaaatgaacagcctgagagccgaagacacggctgtgtattactgtgcgcgagaagattacgatattttgactggttactattacgctatggacgtctggggccaagggaccacggtcaccgtctcc

SEQ ID NO: 126 - protein, 123 aa, Artificial Sequence
  Synthetic
QVQLVESGGGVVQPGRSLRLSCAASGFTFSNFGMHWVRQAPGKGLEWVAVIWFDEIDKYYADSVKGRFTISRDNSKNTLYPQMNSLRAEDTAVYYCAREDYDILTGYYYAMDVWGQGTTVTVS

SEQ ID NO: 127 - DNA, 318 bp, Artificial Sequence
  Synthetic
gacatccagatgacccagtctccatcctccctgtctgcatctgtaggagacagagtcaccatcacttgccgggcaagtcagggcattagaaatgatttaggctggtatcagcagaaaccagggaaagcccctaagcgcctaatctatgctgcatcccgtttgcaaagtggggtcccatcgaggttcagcggcagtggatctgggacagaattcactctcacaatcagcagcctgcagcctgaagattttggaacttattactgtctacagcataatagtcaccccaccttcggccaagggaccaaggtggagatcaaa

SEQ ID NO: 128 - protein, 106 aa, Artificial Sequence
  Synthetic
DIQMTQSPSSLSASVGDRVTITCRASQGIKNDLGWYQQKPGKAPKRLIYAASRLQSGVPSRFSGSGSGTEFTLTISSLQPEDFGTYYCLQHNSHPTFGQGTKVEIK

SEQ ID NO: 129 - DNA, 381 bp, Artificial Sequence
  Synthetic
gaggtgcagctggtggagtcggggggaggcatggtacagcctggggggtccctgagactctcctgtgcagcctctggattcacctccagtaactacgacatgcactgggtccgccaagctacaggaaaaggtctggagtgggtctcaagtattgatactgctggggacacttactatccagactccgtgaagggccgctttatcatctccagagaaaatgccaaaaactccctgtatcttcaaatgaatagcctgagagccggggacacggctgtgtattactgtacaagggagccccgaaattacgaaattttgactggtcactaccactaccacggtatggacatctggggccaagggaccacggtcaccgtctcctca

SEQ ID NO: 130 - protein, 127 aa, Artificial Sequence
  Synthetic
EVQLVESGGGMVQPGGSLRLSCAASGFTSSNYDMHWVRQATGKGLEWVSSIDTAGDTYYPDSVKGRFIISRENAKNSLYLQMNSLRAGDTAVYYCTREPRNYEILTGHYHYHGMDIWGQGTTVTVSS

SEQ ID NO: 131 - DNA, 24 bp, Artificial Sequence
  Synthetic
ggattcacctccagtaactacgac

SEQ ID NO: 132 - protein, 8 aa, Artificial Sequence
  Synthetic
GFTSSNYD

SEQ ID NO: 133 - DNA, 21 bp, Artificial Sequence
  Synthetic
attgatactgctggggacact

SEQ ID NO: 134 - protein, 7 aa, Artificial Sequence
  Synthetic
IDTAGDT

SEQ ID NO: 135 - DNA, 63 bp, Artificial Sequence
  Synthetic
acaagggagccccgaaattacgaaattttgactggtcactaccactaccacggtatggacatc

SEQ ID NO: 136 - protein, 21 aa, Artificial Sequence
  Synthetic
TREPRNYEILTGHYHYHGMDI

SEQ ID NO: 137 - DNA, 324 bp, Artificial Sequence
  Synthetic
gacatccagatgacccagtcgccatcctccctgtctgcatctgtaggagacagagtcaccatcacttgccgggcaagtcaggccattagaaatgatttaggctggtatcagcagaaaccagggaaagcccctaaactcctgatctatactgcattcagtttacagagtggggtcccatcaaggttcagcggcagtaaatctggcacagacttcactctcaccatcagcagcctgcagcctgaagattttgcgacttattactgtctgcaggattacactaatcctcggacgttcggccaagggaccaaggtggagatcaaacga

SEQ ID NO: 138 - protein, 108 aa, Artificial Sequence
  Synthetic
DIQMTQSPSSLSASVGDRVTITCRASQAIRNDLGWYQQKPGKAPKLLIYTAFSLQSGVPSRFSGSKSGTDFTLTISSLQPEDFATYYCLQDYTNPRTFGQGTKVEIKR

SEQ ID NO: 139 - DNA, 18 bp, Artificial Sequence
  Synthetic
caggccattagaaatgat

SEQ ID NO: 140 - protein, 6 aa, Artificial Sequence
  Synthetic
QAIRND

SEQ ID NO: 141 - DNA, 9 bp, Artificial Sequence
  Synthetic
actgcattc

SEQ ID NO: 142 - protein, 3 aa, Artificial Sequence
  Synthetic
TAF

SEQ ID NO: 143 - DNA, 27 bp, Artificial Sequence
  Synthetic
ctgcaggattacactaatcctcggacg

SEQ ID NO: 144 - protein, 9 aa, Artificial Sequence
  Synthetic
LQDYTNPRT

SEQ ID NO: 145 - DNA, 378 bp, Artificial Sequence
  Synthetic
gaggtgcagctggtggagtcggggggaggcatggtacagcctggggggtccctgagactctcctgtgcagcctctggattcacctccagtaactacgacatgcactgggtccgccaagctacaggaaaaggtctggagtgggtctcaagtattgatactgctggggacacttactatccagactccgtgaagggccgctttatcatctccagagaaaatgccaaaaactccctgtatcttcaaatgaatagcctgagagccggggacacggctgtgtattactgtacaagggagccccgaaattacgaaattttgactggtcactaccactaccacggtatggacatctggggccaagggaccacggtcaccgtctcc

SEQ ID NO: 146 - protein, 126 aa, Artificial Sequence
  Synthetic
EVQLVESGGGMVQPGGSLRLSCAASGFTSSNYDMHWVRQATGKGLEWVSSIDTAGDTYYPDSVKGRFIISRENAKNSLYLQMNSLRAGDTAVYYCTREPRNYEILTGHYHYHGMDIWGQGTTVTVS

SEQ ID NO: 147 - DNA, 321 bp, Artificial Sequence
  Synthetic
gccatccagatgacccagtcgccatcctccctgtctgcatctgtaggagacagagtcaccatcacttgccgggcaagtcaggccattagaaatgatttaggctggtatcagcagaaaccagggaaagcccctaaactcctgatctatactgcattcagtttacagagtggggtcccatcaaggttcagcggcagtaaatctggcacagacttcactctcaccatcagcagcctgcagcctgaagattttgcgacttattactgtctgcaggattacactaatcctcggacgttcggccaagggaccaaggtggaaatcaaa

SEQ ID NO: 148 - protein, 107 aa, Artificial Sequence
  Synthetic
AIQMTQSPSSLSASVGDRVTITCRASQAIRNDLGWYQQKPGKAPKLLIYTAFSLQSGVPSRFSGSKSGTDFTLTISSLQPEDFATYYCLQDYTNPRTFGQGTKVEIK

SEQ ID NO: 149 - protein, 345 aa, Artificial Sequence
  Synthetic
QVMDFLFEKWKLYGDQCHHNLSLLPPPTELVCNRTFDKYSCWPDTPANTTANISCPWYLPWHHKVQHRFVFKRCGPDGQWVRGPRGQPWRDASQCQMDGEEIEVQKEVAKMYSSFQVMDKTHTCPPCPAPELLGGPSVFLFPPKPKDTLMISRTPEVTCVVVDVSHEDPEVKFNWYVDGVEVHNAKTKPREEQYNSTYRVVSVLTVLHQDWLNGKEYKCKVSNKALPAPIEKTISKAKGQPREPQVYTLPPSRDELTKNQVSLTCLVKGFYPSDIAVEWESNGQPENNYKTTPPVLDSDGSFFLYSKLTVDKSRWQQGNVFSCSVMHEALHNHYTQKSLSLSPGK

SEQ ID NO: 150 - protein, 348 aa, Artificial Sequence
  Synthetic
QVMDFLFEKWKLYGDQCHHNLSLLPPPTELVCNRTFDKYSCWPDTPANTTANISCPWYLPWHHKVQHRFVFKRCGPDGQWVRGPRGQPWRDASQCQMDGEEIEVQKEVAKMYSSFQVMGPGDKTHTCPPCPAPELLGGPSVFLFPPKPKDTLMISRTPEVTCVVVDVSHEDPEVKFNWYVDGVEVHNAKTKPREEQYNSTYRVVSVLTVLHQDWLNGKEYKCKVSNKALPAPIEKTISKAKGQPREPQVYTLPPSRDELTKNQVSLTCLVKGFYPSDIAVEWESNGQPENNYKTTPPVLDSDGSFFLYSKLTVDKSRWQQGNVFSCSVMHEALHNHYTQKSLSLSPGK

SEQ ID NO: 151 - protein, 146 aa, Artificial Sequence
  Synthetic
QVMDFLFEKWKLYGDQCHHNLSLLPPPTELVCNRTFDKYSCWPDTPANTTANISCPWYLPWHHKVQHRFVFKRCGPDGQWVRGPRGQPWRDASQCQMDGEEIEVQKEVAKMYSSFQVMEQKLISEEDLGGEQKLISEEDLHHHHHH

SEQ ID NO: 152 - protein, 351 aa, Artificial Sequence
  Synthetic
GAPQVMDFLFEKWKLYGDQCHHNLSLLPPPTELVCNRTFDKYSCWPDTPANTTANISCPWYLPWHHKVQHRFVFKRCGPDGQWVRGPRGQPWRDASQCQMDGEELEVQKEVAKMYSSFQVMGPGDKTHTCPPCPAPELLGGPSVFLFPPKPKDTLMISRTPEVTCVVVDVSHEDPEVKFNWYVDGVEVHNAKTKPREEQYNSTYRVVSVLTVLHQDWLNGKEYKCKVSNKALPAPIEKTISKAKGQPREPQVYTLPPSRDELTKNQVSLTCLVKGFYPSDIAVEWESNGQPENNYKTTPPVLDSDGSFFLYSKLTVDKSRWQQGNVFSCSVMHEALHNHYTQKSLSLSPGK

SEQ ID NO: 153 - protein, 477 aa, Homo sapiens
MPPCQPQRPLLLLLLLLACQPQVPSAQVMDFLFEKWKLYGDQCHHNLSLLPPPTELVCNRTFDKYSCWPDTPANTTANISCPWYLPWHHKVQHRFVFKRCGPDGQWVRGPRGQPWRDASQCQMDGEEIEVQKEVAKMYSSFQVMYTVGYSLSLGALLLALAILGGLSKLHCTRNAIHANLFASFVLKASSVLVIDGLLRTRYSQKIGDDLSVSTWLSDGAVAGCRVAAVFMQYGIVANYCWLLVEGLYLHNLLGLATLPERSFFSLYLGIGWGAPMLFVVPWAVVKCLFENVQCWTSNDNMGFWWILRFPVFLAILINFFIFVRIVQLLVAKLRARQMHHTDYKFRLAKSTLTLIPLLGVHEVVFAFVTDEHAQGTLRSAKLFFDLFLSSFQGLLVAVLYCFLNKEVQSELRRRWHRWRLGKVLWEERNTSNHRASSSPGHGPPSKELQFGRGGGSQDSSAETPLAGGLPRLAESPF

SEQ ID NO: 154 - protein, 485 aa, Mus musculus
MALTQLHCPHLLLLLLVLSCLPEAPSAQVMDFLFEKWKLYSDQCHHNLSLLPPPTELVCNRTFDKYSCWPDTPPNTTANISCPWYLPWYHKVQHRLVFKRCGPDGQWVRGPRGQPWRNASQCQLDDEEIEVQKGVAKMYSSQQVMYTVGYSLSLGALLLALVILLGLRKLHCTRNYIHGNLFASFVLKAGSVLVIDWLLKTRYSQKIGDDLSVSVWLSDGAMAGCRVATVIMQYGIIANYCWLLVEGVYLYSLLSLATFSERSFFSLYLGIGWGAPLLFVIPWVVVKCLFENVQCWTSNDNMGFWWILRIPVFLALLINFFIFVHIIHLLVAKLRAHQMHYADYKFRLARSTLTLIPLLGVHEVVFAFVTDEHAQGTLRSTKLFFDLFLSSFQGLLVAVLYCFLNKEVQAELMRRWRQWQEGKALQEERLASSHGSHMAPAGPCHGDPCEKLQLMSAGSSSGTGCVPSMETSLASSLPRLADSPT

SEQ ID NO: 155 - protein, 491 aa, Macaca fascicularis
MAPCQPRRPLLLLLLLLACQPQAPSAQVMDFLFEKWKLYGDQCHHNLSLLPPPTELVCNRTFDKYSCWPDTPANTTANISCPWYLPWHHKVQHRFVFKRCGPDGQWVRGPRGQPWRDASQCQMDGEELEVQKEVAKMYSSFQVMYTVGYSLSLGALLLALAILGGISKLHCTRNAIHANLFVSFVLKASSVLVIDGLLRTRYSQKIGDDLSVSIWLSDGAVAGCRVAAVFMQYGVVANYCWLLVEGLYLHNLLGLATLPERSFFSLYLGIGWGAPMLFIIPWVVVRCLFENIQCWTSNDNMGFWWILRFPVFLAILINFFIFIRIVHLLVAKLRAREMHHTDYKFRLAKSTLTLIPLLGVHEVVFAFVTDEHAQGTLRFAKLFFDLFLSSFQGLLVAVLYCFLNKEVQSELRRHWHRWRLGKVLQEERGTSNHKAPSAPGQGLPGKKLQSGRDGGSQDSSAEIPLAGGLPRLAESPFSTLLGPQLGLDSGT

SEQ ID NO: 156 - protein, 485 aa, Rattus norvegicus
MVLTQLHCPYLLLLLVVLSCLPKAPSAQVMDFLFEKWKLYSDQCHHNLSLLPPPTELVCNRTFDKYSCWPDTPPNTTANISCPWYLPWYHKVQHRLVFKRCGPDGQWVRGPRGQSWRDASQCQMDDDEIEVQKGVAKMYSSYQVMYTVGYSLSLGALLLALVILLGLRKLHCTRNYIHGNLFASFVLKAGSVLVIDWLLKTRYSQKIGDDLSVSVWLSDGAVAGCRVATVIMQYGIIANYCWLLVEGVYLYSLLSITTFSEKSFFSLYLCIGWGSPLLFVIPWVVVKCLFENVQCWTSNDNMGFWWILRIPVLLAILINFFIFVRIIHLLVAKLRAHQMHYADYKFRLARSTLTLIPLLGVHEVVFAFVTDEHAQGTLRSTKLFFDLFFSSFQGLLVAVLYCFLNKEVQAELLRRWRRWQEGKALQEERMASSHGSHMAPAGTCHGDPCEKLQLMSAGSSSGTGCEPSAKTSLASSLPRLADSPT

SEQ ID NO: 157 - DNA, 1434 bp, Homo sapiens
atgcccccctgccagccacagcgacccctgctgctgttgctgctgctgctggcctgccagccacaggtcccctccgctcaggtgatggacttcctgtttgagaagtggaagctctacggtgaccagtgtcaccacaacctgagcctgctgccccctcccacggagctggtgtgcaacagaaccttcgacaagtattcctgctggccggacacccccgccaataccacggccaacatctcctgcccctggtacctgccttggcaccacaaagtgcaacaccgcttcgtgttcaagagatgcgggcccgacggtcagtgggtgcgtggaccccgggggcagccttggcgtgatgcctcccagtgccagatggatggcgaggagattgaggtccagaaggaggtggccaagatgtacagcagcttccaggtgatgtacacagtgggctacagcctgtccctgggggccctgctcctcgccttggccatcctggggggcctcagcaagctgcactgcacccgcaatgccatccacgcgaatctgtttgcgtccttcgtgctgaaagccagctccgtgctggtcattgatgggctgctcaggacccgctacagccagaaaattggcgacgacctcagtgtcagcacctggctcagtgatggagcggtggctggctgccgtgtggccgcggtgttcatgcaatatggcatcgtggccaactactgctggctgctggtggagggcctgtacctgcacaacctgctgggcctggccaccctccccgagaggagcttcttcagcctctacctgggcatcggctggggtgcccccatgctgttcgtcgtcccctgggcagtggtcaagtgtctgttcgagaacgtccagtgctggaccagcaatgacaacatgggcttctggtggatcctgcggttccccgtcttcctggccatcctgatcaacttcttcatcttcgtccgcatcgttcagctgctcgtggccaagctgcgggcacggcagatgcaccacacagactacaagttccggctggccaagtccacgctgaccctcatccctctgctgggcgtccacgaagtggtctttgccttcgtgacggacgagcacgcccagggcaccctgcgctccgccaagctcttcttcgacctcttcctcagctccttccagggcctgctggtggctgtcctctactgcttcctcaacaaggaggtgcagtcggagctgcggcggcgttggcaccgctggcgcctgggcaaagtgctatgggaggagcggaacaccagcaaccacagggcctcatcttcgcccggccacggccctcccagcaaggagctgcagtttgggaggggtggtggcagccaggattcatctgcggagacccccttggctggtggcctccctagattggctgagagccccttctga

SEQ ID NO: 158 - DNA, 354 bp, Homo sapiens
caggtgatggacttcctgtttgagaagtggaagctctacggtgaccagtgtcaccacaacctgagcctgctgccccctcccacggagctggtgtgcaacagaaccttcgacaagtattcctgctggccggacacccccgccaataccacggccaacatctcctgcccctggtacctgccttggcaccacaaagtgcaacaccgcttcgtgttcaagagatgcgggcccgacggtcagtgggtgcgtggaccccgggggcagccttggcgtgatgcctcccagtgccagatggatggcgaggagattgaggtccagaaggaggtggccaagatgtacagcagcttccaggtgatg

SEQ ID NO: 159 - protein, 118 aa, Homo sapiens
QVMDFLFEKWKLYGDQCHHNLSLLPPPTELVCNRTFDKYSCWPDTPANTTANISCPWYLPWHHKVQHRFVFKRCGPDGQWVRGPRGQPWRDASQCQMDGEEIEVQKEVAKMYSSFQVM

SEQ ID NO: 160 - DNA, 24 bp, Artificial Sequence
  Synthetic
ggattcacctttaacaactatgcc

SEQ ID NO: 161 - protein, 8 aa, Artificial Sequence
  Synthetic
GFTFNNYA

SEQ ID NO: 162 - DNA, 24 bp, Artificial Sequence
  Synthetic
attagtggtagcggtggtactaca

SEQ ID NO: 163 - protein, 8 aa, Artificial Sequence
  Synthetic
ISGSGGTT

SEQ ID NO: 164 - DNA, 33 bp, Artificial Sequence
  Synthetic
gcgaaagattctaactggggaaatttcgatctc

SEQ ID NO: 165 - protein, 11 aa, Artificial Sequence
  Synthetic
AKDSNWGNFDL

SEQ ID NO: 166 - DNA, 36 bp, Artificial Sequence
  Synthetic
cagagtgttttatacaggtccaacaataggaacttc

SEQ ID NO: 167 - protein, 12 aa, Artificial Sequence
  Synthetic
QSVLYRSNNRNF

SEQ ID NO: 168 - DNA, 9 bp, Artificial Sequence
  Synthetic
tgggcatct

SEQ ID NO: 169 - protein, 3 aa, Artificial Sequence
  Synthetic
WAS

SEQ ID NO: 170 - DNA, 27 bp, Artificial Sequence
  Synthetic
caacaatattatactactccgtacact

SEQ ID NO: 171 - protein, 9 aa, Artificial Sequence
  Synthetic
QQYYTTPYT

SEQ ID NO: 172 - DNA, 354 bp, Artificial Sequence
  Synthetic
gaggtgcagctggtggagtctgggggaggcttggtacagcctggggggtccctgagactctcctgtgcagcctctggattcacctttaacaactatgccatgaactgggtccgccaggctccaggaaagggactggactgggtctcaactattagtggtagcggtggtactacaaactacgcagactccgtgaagggccgtttcattatttcccgagacagttccaaacacacgctgtatctgcaaatgaacagcctgagagccgaggacacggccgtatattactgtgcgaaagattctaactggggaaatttcgatctctggggccgtggcaccctggtcactgtctcctca

SEQ ID NO: 173 - protein, 118 aa, Artificial Sequence [sequence omitted]

SEQ ID NO: 174 - DNA, 339 bp, Artificial Sequence
  Synthetic
gacatcgtgatgacccagtctccagactccctggctgtgtctctgggcgagagggccaccatcaactgcaagtccagccagagtgttttatacaggtccaacaataggaacttcttaggttggtaccagcagaaaccagggcagcctcctaatctactcatttactgggcatctacccgggaatccggggtccctgaccgattcagtggcagcgggtctgggacagatttcactctcaccatcagcagcctgcaggctgaagatgtggcagtttattactgtcaacaatattatactactccgtacacttttggccaggggaccaagctggagatcaaa

SEQ ID NO: 175 - protein, 113 aa, Artificial Sequence [sequence omitted]

SEQ ID NO: 176 - DNA, 381 bp, Artificial Sequence
  Synthetic
gagatgcaactggtggagtctgggggaggcttggtccagcctggggggtccctgagactctcctgtgcagcctctggattcacctttagtagtcactggatgaagtgggtccgccaggctccagggaaggggctggagtgggtggccaacataaaccaagatggaagtgagaaatactatgtggactctgtgaagggccgattcaccatctccagagacaacgccaagaactcactgtttctgcaaatgaacagcctgagagccgaggacacggctgtgtattactgtgcgagagatattgtactaatggtctatgatatggactactactactacggtatggacgtctggggccaagggaccacggtcaccgtctcctca

SEQ ID NO: 177 - protein, 127 aa, Artificial Sequence
  Synthetic
EMQLVESGGGLVQPGGSLRLSCAASGFTFSSHWMKWVRQAPGKGLEWVANINQDGSEKYYVDSVKGRFTISRDNAKNSLFLQMNSLRAEDTAVYYCARDIVLMVYDMDYYYYGMDVWGQGTTVTVSS

SEQ ID NO: 178 - DNA, 24 bp, Artificial Sequence
  Synthetic
ggattcacctttagtagtcactgg

SEQ ID NO: 179 - protein, 8 aa, Artificial Sequence
  Synthetic
GFTFSSHW

SEQ ID NO: 180 - DNA, 24 bp, Artificial Sequence
  Synthetic
ataaaccaagatggaagtgagaaa

SEQ ID NO: 181 - protein, 8 aa, Artificial Sequence
  Synthetic
INQDGSEK

SEQ ID NO: 182 - DNA, 60 bp, Artificial Sequence
  Synthetic
gcgagagatattgtactaatggtctatgatatggactactactactacggtatggacgtc

SEQ ID NO: 183 - protein, 20 aa, Artificial Sequence
  Synthetic
ARDIVLMVYDMDYYYYGMDV

SEQ ID NO: 184 - DNA, 336 bp, Artificial Sequence
  Synthetic
gatattgtgatgactcagtctccactctccctgcccgtcacccctggagagccggcctccatctcctgcaggtctagtcagagcctcctgcatagtaatggaaacaactatttggattggtacctgcagaagccagggcagtctccacagctcctgatctatttgggttctaatcgggcctccggggtccctgacaggttcagtggcagtggatcaggcacagattttacactgaaaatcagcagagtggaggctgaggatgttggggtttattactgcatgcaaactctacaaactccgctcactttcggcggagggaccaaggtggagatcaaa

SEQ ID NO: 185 - protein, 112 aa, Artificial Sequence
  Synthetic
DIVMTQSPLSLPVTPGEPASISCRSSQSLLHSNGNNYLDWYLQKPGQSPQLLIYLGSNRASGVPDRFSGSGSGTDFTLKISRVEAEDVGVYYCMQTLQTPLTFGGGTKVEIK

SEQ ID NO: 186 - DNA, 33 bp, Artificial Sequence
  Synthetic
cagagcctcctgcatagtaatggaaacaactat

SEQ ID NO: 187 - protein, 11 aa, Artificial Sequence
  Synthetic
QSLLHSNGNNY

SEQ ID NO: 188 - DNA, 9 bp, Artificial Sequence
  Synthetic
ttgggttct

SEQ ID NO: 189 - protein, 3 aa, Artificial Sequence
  Synthetic
LGS

SEQ ID NO: 190 - DNA, 27 bp, Artificial Sequence
  Synthetic
atgcaaactctacaaactccgctcact

SEQ ID NO: 191 - protein, 9 aa, Artificial Sequence
  Synthetic
MQTLQTPLT

SEQ ID NO: 192 - DNA, 2076 bp, Homo sapiens
atgggcaccgtcagctccaggcggtcctggtggccgctgccactgctgctgctgctgctgctgctcctgggtcccgcgggcgcccgtgcgcaggaggacgaggacggcgactacgaggagctggtgctagccttgcgttccgaggaggacggcctggccgaagcacccgagcacggaaccacagccaccttccaccgctgcgccaaggatccgtggaggttgcctggcacctacgtggtggtgctgaaggaggagacccacctctcgcagtcagagcgcactgcccgccgcctgcaggcccaggctgcccgccggggatacctcaccaagatcctgcatgtcttccatggccttcttcctggcttcctggtgaagatgagtggcgacctgctggagctggccttgaagttgccccatgtcgactacatcgaggaggactcctctgtctttgcccagagcatcccgtggaacctggagcggattacccctccacggtaccgggcggatgaataccagccccccgacggaggcagcctggtggaggtgtatctcctagacaccagcatacagagtgaccaccgggaaatcgagggcagggtcatggtcaccgacttcgagaatgtgcccgaggaggacgggacccgcttccacagacaggccagcaagtgtgacagtcatggcacccacctggcaggggtggtcagcggccgggatgccggcgtggccaagggtgccagcatgcgcagcctgcgcgtgctcaactgccaagggaagggcacggttagcggcaccctcataggcctggagtttattcggaaaagccagctggtccagcctgtggggccactggtggtgctgctgcccctggcgggtgggtacagccgcgtcctcaacgccgcctgccagcgcctggcgagggctggggtcgtgctggtcaccgctgccggcaacttccgggacgatgcctgcctctactccccagcctcagctcccgaggtcatcacagttggggccaccaatgcccaggaccagccggtgaccctggggactttggggaccaactttggccgctgtgtggacctctttgccccaggggaggacatcattggtgcctccagcgactgcagcacctgctttgtgtcacagagtgggacatcacaggctgctgcccacgtggctggcattgcagccatgatgctgtctgccgagccggagctcaccctggccgagttgaggcagagactgatccacttctctgccaaagatgtcatcaatgaggcctggttccctgaggaccagcgggtactgacccccaacctggtggccgccctgccccccagcacccatggggcaggttggcagctgttttgcaggactgtgtggtcagcacactcggggcctacacggatggccacagccatcgcccgctgcgccccagatgaggagctgctgagctgctccagtttctccaggagtgggaagcggcggggcgagcgcatggaggcccaagggggcaagctggtctgccgggcccacaacgcttttgggggtgagggtgtctacgccattgccaggtgctgcctgctaccccaggccaactgcagcgtccacacagctccaccagctgaggccagcatggggacccgtgtccactgccaccaacagggccacgtcctcacaggctgcagctcccactgggaggtggaggaccttggcacccacaagccgcctgtgctgaggccacgaggtcagcccaaccagtgcgtgggccacagggaggccagcatccacgcttcctgctgccatgccccaggtctggaatgcaaagtcaaggagcatggaatcccggcccctcaggagcaggtgaccgtggcctgcgaggagggctggaccctgactggctgcagtgccctccctgggacctcccacgtcctgggggcctacgccgtagacaacacgtgtgtagtcaggagccgggacgtcagcactacaggcagcaccagcgaagaggccgtgacagccgttgccatctgctgccggagccggcacctggcgcaggcctcccaggagctccag

SEQ ID NO: 193 - protein, 692 aa, Homo sapiens
MGTVSSRRSWWPLPLLLLLLLLLGPAGARAQEDEDGDYEELVLALRSEEDGLAEAPEHGTTATFHRCAKDPWRLPGTYVVVLKEETHLSQSERTARRLQAQAARRGYLTKILHVFHGLLPGFLVKMSGDLLELALKLPHVDYIEEDSSVFAQSIPWNLERITPPRYRADEYQPPDGGSLVEVYLLDTSIQSDHREIEGRVMVTDFENVPEEDGTRFHRQASKCDSHGTHLAGVVSGRDAGVAKGASMRSLRVLNCQGKGTVSGTLIGLEFIRKSQLVQPVGPLVVLLPLAGGYSRVLNAACQRLARAGVVLVTAAGNFRDDACLYSPASAPEVITVGATNAQDQPVTLGTLGTNFGRCVDLFAPGEDIIGASSDCSTCFVSQSGTSQAAAHVAGIAAMMLSAEPELTLAELRQRLIHFSAKDVINEAWFPEDQRVLTPNLVAALPPSTHGAGWQLFCRTVWSAHSGPTRMATAIARCAPDEELLSCSSFSRSGKRRGERMEAQGGKLVCRAHNAFGGEGVYAIARCCLLPQANCSVHTAPPAEASMGTRVHCHQQGHVLTGCSSHWEVEDLGTHKPPVLRPRGQPNQCVGHREASIHASCCHAPGLECKVKEHGIPAPQEQVTVACEEGWTLTGCSALPGTSHVLGAYAVDNTCVVRSRDVSTTGSTSEEAVTAVAICCRSRHLAQASQELQ

SEQ ID NO: 194 - protein, 115 aa, Artificial Sequence
  Synthetic
EVQLVQSGGGLVHPGGSLRLSCAGSGFTFSRNAMFWVRQAPGKGLEWVSGIGTGGATNYADSVKGRFTISRDNAKNSLYLQMNSLRAEDMAVYYCARGRYYFDYWGQGTLVTVSS

SEQ ID NO: 195 - protein, 8 aa, Artificial Sequence
  Synthetic
GFTFSRNA

SEQ ID NO: 196 - protein, 7 aa, Artificial Sequence
  Synthetic
IGTGGAT

SEQ ID NO: 197 - protein, 9 aa, Artificial Sequence
  Synthetic
ARGRYYFDY

SEQ ID NO: 198 - protein, 109 aa, Artificial Sequence
  Synthetic
EIVLTQSPGTLSLSPGERATLSCRASQSVSSSYLAWYQQKPGQAPRLLIFGASSRATGIPDRFSGSGSGTDFTLTISRLEPEDFAVYYCQQYGSSPPWTFGQGTKVEIK

SEQ ID NO: 199 - protein, 7 aa, Artificial Sequence
  Synthetic
QSVSSSY

SEQ ID NO: 200 - protein, 3 aa, Artificial Sequence
  Synthetic
GAS

SEQ ID NO: 201 - protein, 10 aa, Artificial Sequence
  Synthetic
QQYGSSPPWT

SEQ ID NO: 202 - protein, 8 aa, Artificial Sequence
  Synthetic
  VARIANT (1)...(1): Xaa = Gly
  VARIANT (2)...(2): Xaa = Phe
  VARIANT (3)...(3): Xaa = Thr
  VARIANT (4)...(4): Xaa = Phe or Ser
  VARIANT (5)...(5): Xaa = Ser
  VARIANT (6)...(6): Xaa = Ser or Asn
  VARIANT (7)...(7): Xaa = Tyr or Phe
  VARIANT (8)...(8): Xaa = Asp, Leu, or Gly
XXXXXXXX

SEQ ID NO: 203 - protein, 8 aa, Artificial Sequence
  Synthetic
  VARIANT (1)...(1): Xaa = Ile
  VARIANT (2)...(2): Xaa = Ser, Gln, Asp, or Trp
  VARIANT (3)...(3): Xaa = Ser, Glu, Thr, or Phe
  VARIANT (4)...(4): Xaa = Asp or Ala
  VARIANT (5)...(5): Xaa = Gly or Glu
  VARIANT (6)...(6): Xaa = Arg, Ile, or absent
  VARIANT (7)...(7): Xaa = Asp or Glu
  VARIANT (8)...(8): Xaa = Lys or Thr
XXXXXXXX

SEQ ID NO: 204 - protein, 21 aa, Artificial Sequence
  Synthetic
  VARIANT (1)...(1): Xaa = Ala or Thr
  VARIANT (2)...(2): Xaa = Lys or Arg
  VARIANT (3)...(3): Xaa = Glu
  VARIANT (4)...(4): Xaa = Met, Pro, Gly, or Asp
  VARIANT (5)...(5): Xaa = Val, Ser, Lys, Arg, or absent
  VARIANT (6)...(6): Xaa = Tyr, His, Asn, or absent
  VARIANT (7)...(7): Xaa = Tyr
  VARIANT (8)...(8): Xaa = Asp or Glu
  VARIANT (9)...(9): Xaa = Ile
  VARIANT (10)...(10): Xaa = Leu
  VARIANT (11)...(11): Xaa = Thr
  VARIANT (12)...(12): Xaa = Gly
  VARIANT (13)...(13): Xaa = Tyr, Asp, or His
  VARIANT (14)...(14): Xaa = His, Asp, Tyr, or absent
  VARIANT (15)...(15): Xaa = Asn, Tyr, His, or absent
  VARIANT (16)...(16): Xaa = Tyr
  VARIANT (17)...(17): Xaa = Tyr or His
  VARIANT (18)...(18): Xaa = Gly or Ala
  VARIANT (19)...(19): Xaa = Met
  VARIANT (20)...(20): Xaa = Asp
  VARIANT (21)...(21): Xaa = Val or Ile
XXXXXXXXXXXXXXXXXXXXX

SEQ ID NO: 205 - protein, 6 aa, Artificial Sequence
  Synthetic
  VARIANT (1)...(1): Xaa = Gln
  VARIANT (2)...(2): Xaa = Gly or Ala
  VARIANT (3)...(3): Xaa = Ile
  VARIANT (4)...(4): Xaa = Asn or Arg
  VARIANT (5)...(5): Xaa = Asn
  VARIANT (6)...(6): Xaa = Tyr or Asp
XXXXXX

SEQ ID NO: 206 - protein, 3 aa, Artificial Sequence
  Synthetic
  VARIANT (1)...(1): Xaa = Thr or Ala
  VARIANT (2)...(2): Xaa = Ala or Thr
  VARIANT (3)...(3): Xaa = Ser or Phe
XXX

SEQ ID NO: 207 - protein, 9 aa, Artificial Sequence
  Synthetic
  VARIANT (1)...(1): Xaa = Gln or Leu
  VARIANT (2)...(2): Xaa = Gln
  VARIANT (3)...(3): Xaa = Tyr, His, or Asp
  VARIANT (4)...(4): Xaa = Asn or Tyr
  VARIANT (5)...(5): Xaa = Thr or Ser
  VARIANT (6)...(6): Xaa = Tyr, Asn, or His
  VARIANT (7)...(7): Xaa = Pro
  VARIANT (8)...(8): Xaa = Leu, Phe, Arg, or absent
  VARIANT (9)...(9): Xaa = Thr
XXXXXXXXX